European Patent Application EP 4 484 573 A2, published January 1, 2025. Title: COMPOSITIONS AND METHODS FOR CHROMATIN AND GENE EXPRESSION ANALYSIS IN SINGLE CELLS. Applicant: Agilent Technologies, Inc. Application US 18/335,896, filed June 15, 2023. The sequence listing filed with the application follows.

SEQUENCE LISTING (19 sequences)

SEQ ID NO: 1 - DNA, 63 bp, synthetic construct
  source 1..63: mol_type = other DNA
ggagaattgtaatacgactcactatagggagacgcgtgatcacgnnnnnnnnnnnnnnntgtg

SEQ ID NO: 2 - DNA, 60 bp, synthetic construct
  source 1..60: mol_type = other DNA
ggagaattgtaatacgactcactatagggagacgcgtgatcacgnnnnnnnnnnnnnnnt

SEQ ID NO: 3 - DNA, 62 bp, synthetic construct
  source 1..62: mol_type = other DNA
aaannnnnnnnnnnnnnncgtgatcacgcgtctccctatagtgagtcgtattacaattctcc

SEQ ID NO: 4 - DNA, 47 bp, synthetic construct
  source 1..47: mol_type = other DNA
ggagaattgtaatacgactcactatagggagacgcgtgatcacgaca

SEQ ID NO: 5 - DNA, 44 bp, synthetic construct
  source 1..44: mol_type = other DNA
cgtgatcacgcgtctccctatagtgagtcgtattacaattctcc

SEQ ID NO: 6 - skipped

SEQ ID NO: 7 - DNA, 28 bp, synthetic construct
  source 1..28: mol_type = other DNA
aaannnnnnnnnnnnnnntcctcattgt

SEQ ID NO: 8 - DNA, 18 bp, synthetic construct
  source 1..18: mol_type = other DNA
tagggagacgcgtgatca

SEQ ID NO: 9 - DNA, 18 bp, synthetic construct
  source 1..18: mol_type = other DNA
tagggagacgcgtgagtt

SEQ ID NO: 10 - DNA, 34 bp, synthetic construct
  source 1..34: mol_type = other DNA
gcgccattgaccaggattttcccccccccccccc

SEQ ID NO: 11 - DNA, 21 bp, synthetic construct
  source 1..21: mol_type = other DNA
gcgccattgaccaggattttc

SEQ ID NO: 12 - DNA, 20 bp, synthetic construct
  source 1..20: mol_type = other DNA
tccttagctgttgcagaaat

SEQ ID NO: 13 - DNA, 20 bp, synthetic construct
  source 1..20: mol_type = other DNA
cgttcagttgatgcagagtg

SEQ ID NO: 14 - DNA, 20 bp, synthetic construct
  source 1..20: mol_type = other DNA
agaagcagcttcaaacctgc

SEQ ID NO: 15 - DNA, 20 bp, synthetic construct
  source 1..20: mol_type = other DNA
aagttagctttacagtgggc

SEQ ID NO: 16 - DNA, 20 bp, synthetic construct
  source 1..20: mol_type = other DNA
ggtgttggttctcttaatct

SEQ ID NO: 17 - DNA, 20 bp, synthetic construct
  source 1..20: mol_type = other DNA
atttagttggggcatttcac

SEQ ID NO: 18 - DNA, 20 bp, synthetic construct
  source 1..20: mol_type = other DNA
ttatggtgggtcatacggta

SEQ ID NO: 19 - DNA, 20 bp, synthetic construct
  source 1..20: mol_type = other DNA
tagtgtaaggagtatggggg